European Patent Specification EP 3 969 000 B1, published August 30, 2023. Title: BCL-2 INHIBITORS FOR USE IN THE TREATMENT OF A BCL-2 MEDIATED CANCER CARRYING THE GLY101VAL MUTATION. Applicant: Les Laboratoires Servier and Novartis AG. The sequence listing filed with the application follows.

SEQUENCE LISTING (8 sequences)

SEQ ID NO: 1 - protein, 21 aa, Homo sapiens
QWAREIGAQLRRMADDLNAQY

SEQ ID NO: 2 - protein, 221 aa, Homo sapiens
MGHHHHHHHHSAGLVPRGSMAHAGRTGYDNREIVMKYIHYKLSQRGYEWDAGDVGAAPPGAAPAPGIFSSQPGHTPHPAASRDPVARTSPLQTPAAPGAAAGPALSPVPPVVHLTLRQAGDDFSRRYRRDFAEMSSQLHLTPFTARGRFATVVEELFRDGVNWGRIVAFFEFGGVMCVESVNREMSPLVDNIALWMTEYLNRHLHTWIQDNGGWDAFVELY

SEQ ID NO: 3 - protein, 221 aa, Homo sapiens
MGHHHHHHHHSAGLVPRGSMAHAGRTGYDNREIVMKYIHYKLSQRGYEWDAGDVGAAPPGAAPAPGIFSSQPGHTPHPAASRDPVARTSPLQTPAAPGAAAGPALSPVPPVVHLTLRQAVDDFSRRYRRDFAEMSSQLHLTPFTARGRFATVVEELFRDGVNWGRIVAFFEFGGVMCVESVNREMSPLVDNIALWMTEYLNRHLHTWIQDNGGWDAFVELY

SEQ ID NO: 4 - protein, 221 aa, homo sapiens
MGHHHHHHHHSAGLVPRGSMAHAGRTGYDNREIVMKYIHYKLSQRGYEWDAGDVGAAPPGAAPAPGIFSSQPGHTPHPAASRDPVARTSPLQTPAAPGAAAGPALSPVPPVVHLTLRQAGDYFSRRYRRDFAEMSSQLHLTPFTARGRFATVVEELFRDGVNWGRIVAFFEFGGVMCVESVNREMSPLVDNIALWMTEYLNRHLHTWIQDNGGWDAFVELY

SEQ ID NO: 5 - protein, 221 aa, Homo sapiens
MGHHHHHHHHSAGLVPRGSMAHAGRTGYDNREIVMKYIHYKLSQRGYEWDAGDVGAAPPGAAPAPGIFSSQPGHTPHPAASRDPVARTSPLQTPAAPGAAAGPALSPVPPVVHLTLRQAGDVFSRRYRRDFAEMSSQLHLTPFTARGRFATVVEELFRDGVNWGRIVAFFEFGGVMCVESVNREMSPLVDNIALWMTEYLNRHLHTWIQDNGGWDAFVELY

SEQ ID NO: 6 - protein, 221 aa, Homo sapiens
MGHHHHHHHHSAGLVPRGSMAHAGRTGYDNREIVMKYIHYKLSQRGYEWDAGDVGAAPPGAAPAPGIFSSQPGHTPHPAASRDPVARTSPLQTPAAPGAAAGPALSPVPPVVHLTLRQAGDEFSRRYRRDFAEMSSQLHLTPFTARGRFATVVEELFRDGVNWGRIVAFFEFGGVMCVESVNREMSPLVDNIALWMTEYLNRHLHTWIQDNGGWDAFVELY

SEQ ID NO: 7 - protein, 221 aa, Homo sapiens
MGHHHHHHHHSAGLVPRGSMAHAGRTGYDNREIVMKYIHYKLSQRGYEWDAGDVGAAPPGAAPAPGIFSSQPGHTPHPAASRDPVARTSPLQTPAAPGAAAGPALSPVPPVVHLTLRQAGDDFSRRYRRDFAEMSSQLHLTPFTARGLFATVVEELFRDGVNWGRIVAFFEFGGVMCVESVNREMSPLVDNIALWMTEYLNRHLHTWIQDNGGWDAFVELY

SEQ ID NO: 8 - protein, 221 aa, Homo sapiens
MGHHHHHHHHSAGLVPRGSMAHAGRTGYDNREIVMKYIHYKLSQRGYEWDAGDVGAAPPGAAPAPGIFSSQPGHTPHPAASRDPVARTSPLQTPAAPGAAAGPALSPVPPVVHLTLRQAGDDFSRRYRRDFGEMSSQLHLTPFTARGRFATVVEELFRDGVNWGRIVAFFEFGGVMCVESVNREMSPLVDNIALWMTEYLNRHLHTWIQDNGGWDAFVELY